European Patent Application EP 4 778 388 A1, published July 22, 2026. Title: Sunflower plants with upward flower stem. Applicant: タキイ種苗株式会社. Application JP. The sequence listing filed with the application follows.

SEQUENCE LISTING (27 sequences)

SEQ ID NO: 1 - DNA, 201 bp, Helianthus annuus
  source 1..201: mol_type = genomic DNA
agtataaacacgaatcggaaccgaaagtcttgtaaatcgactttttcgtagactatcgattcggatccgtgcatgcatgtttgagatctgtattggagccaatttttgaccatttttattttagtataactttctggaatttttgatacttgagtctatgcttagccgattcatttgcatgtttccgatttatgcttaaag

SEQ ID NO: 2 - DNA, 400 bp, Helianthus annuus
  source 1..400: mol_type = genomic DNA
ctacgacgcccacttgaatatgttttattatattcttcgcaaaacctatcgacgaacccattcatttttcgccacttagatgacaccgagttgatatctcgatacgggccttggtccattagctcaaggaacttcgccaaaaccgcattccaaaacccctcacccatttgattattacctacaaaatatgttacaaaaaataaaaaaaaaaactaatactacaaaatataaacttaaaaaaaaagttattgttacgaaccttttatcgggtgtgtagacatgcctatgtaagcgttcgctaaggcttcttcatcgagttgcgtctacggtttcgcctttggtttggacggttgctcacccaccacttgcttgccttttcttcgtttgcctttttgcggtt

SEQ ID NO: 3 - DNA, 201 bp, Helianthus annuus
  source 1..201: mol_type = genomic DNA
tttttgactaattaattagtcataaagactagtatcctccacactaacttatttttgcatacacacatcaaaagttatcttacaaatttcgaaattcaccttacaccttaaaatttatcctacacaactcgtaatgtatcttacacaactcgtaatttatcatacactttaaattattttatttcatttttttgaaaaaaa

SEQ ID NO: 4 - DNA, 201 bp, Helianthus annuus
  source 1..201: mol_type = genomic DNA
cgtttatattacagattatgcataaatcgcaaaaatagctttctgttgactttttaagtacgcgtttgactcgacatttgaactagttagagtggtgatcctagggaaccctttcagaggtttattacccacataaataccaacacataaccacttttgattcgacaagtgactgagccattaaggatttatcttgaagtc

SEQ ID NO: 5 - DNA, 201 bp, Helianthus annuus
  source 1..201: mol_type = genomic DNA
gactaatttcatgcctgccttcaaaatggmaaaagaaactaattggaaawttttgtgtttatatyttgtaataatatttgtgcaaaaaggttcatgccttgtaatctatctcttatactaaagcaaaataatgttgactatttgactatgatgtggcagtgctacwtattcagagaattgkgaattrggcggcatttgttt

SEQ ID NO: 6 - DNA, 201 bp, Helianthus annuus
  source 1..201: mol_type = genomic DNA
ctccatggcgtgtaacaatttctctcatgtaaatttcagccaacttgctcgtgttatctttctttcagataggtaagaagtgcgcagatttcgttaatcgatccactattacccaaatagtgtcatggcctcttggtgttctaggaaactttgtaataaaatccatggagatttgttcccatttccacttgggaatttctg

SEQ ID NO: 7 - DNA, 201 bp, Helianthus annuus
  source 1..201: mol_type = genomic DNA; note = n is t or a
agtataaacacgaatcggaaccgaaagtcttgtaaatcgactttttcgtagactatcgattcggatccgtgcatgcatgtttgagatctgtattggagccnatttttgaccatttttattttagtataactttctggaatttttgatacttgagtctatgcttagccgattcatttgcatgtttccgatttatgcttaaag

SEQ ID NO: 8 - DNA, 389 bp, Helianthus annuus
  source 1..389: mol_type = genomic DNA; note = n is taaaaaaaaaaaa or taaaaaaaaaaa
ctacgacgcccacttgaatatgttttattatattcttcgcaaaacctatcgacgaacccattcatttttcgccacttagatgacaccgagttgatatctcgatacgggccttggtccattagctcaaggaacttcgccaaaaccgcattccaaaacccctcacccatttgattattacctacaaaatatgttacaaaaaanctaatactacaaaatataaacttaaaaaaaaagttattgttacgaaccttttatcgggtgtgtagacatgcctatgtaagcgttcgctaaggcttcttcatcgagttgcgtctacggtttcgcctttggtttggacggttgctcacccaccacttgcttgccttttcttcgtttgcctttttgcggtt

SEQ ID NO: 9 - DNA, 201 bp, Helianthus annuus
  source 1..201: mol_type = genomic DNA; note = n is c or t
tttttgactaattaattagtcataaagactagtatcctccacactaacttatttttgcatacacacatcaaaagttatcttacaaatttcgaaattcaccntacaccttaaaatttatcctacacaactcgtaatgtatcttacacaactcgtaatttatcatacactttaaattattttatttcatttttttgaaaaaaa

SEQ ID NO: 10 - DNA, 201 bp, Helianthus annuus
  source 1..201: mol_type = genomic DNA; note = n is a or c
cgtttatattacagattatgcataaatcgcaaaaatagctttctgttgactttttaagtacgcgtttgactcgacatttgaactagttagagtggtgatcntagggaaccctttcagaggtttattacccacataaataccaacacataaccacttttgattcgacaagtgactgagccattaaggatttatcttgaagtc

SEQ ID NO: 11 - DNA, 201 bp, Helianthus annuus
  source 1..201: mol_type = genomic DNA; note = n is a or g
gactaatttcatgcctgccttcaaaatggmaaaagaaactaattggaaawttttgtgtttatatyttgtaataatatttgtgcaaaaaggttcatgccttntaatctatctcttatactaaagcaaaataatgttgactatttgactatgatgtggcagtgctacwtattcagagaattgkgaattrggcggcatttgttt

SEQ ID NO: 12 - DNA, 201 bp, Helianthus annuus
  source 1..201: mol_type = genomic DNA; note = n is g or a
ctccatggcgtgtaacaatttctctcatgtaaatttcagccaacttgctcgtgttatctttctttcagataggtaagaagtgcgcagatttcgttaatcgntccactattacccaaatagtgtcatggcctcttggtgttctaggaaactttgtaataaaatccatggagatttgttcccatttccacttgggaatttctg

SEQ ID NO: 13 - DNA, 855 bp, Helianthus annuus
  source 1..855: mol_type = genomic DNA; note = Insertion sequence
cagtggcggacccaagaatttttccatgggggtgcgaaacatttttaaaaattttaggcccctaggtatataagtaaaaaaatcggttcgtatcgggtcggttcgggtcgggtcatgtaaaacaaaagaaattgcgccataacgtccctactcatggtttctatcacaaacaaattgatgcataagtttatcgctccataaaataatgtttcaattttaattttcaaccctagaaatcgtgtgtaatcagcctaaaaattatctaaacaacataatcaccctaaaaatcatctaaacaaccataaacatcgtcaaaacacatgaaatttcaaacctatttaagaattttgttaccctttggtgtcggacggcggtggttcgcggctgctgatgacgtgctgttgtggtcgatgatcgcttgtaggagacgacccaagagagggagggcgggatgaattctaagggactattgggcttattttaattattatactttgaacttaggttgagtttggttaatgggctagtaattagtgggctaattatgtttaatgaaatagtgggttaaggtattgggtatttgggttaagttgggtagtataagtttatataatttagatagtttttttaattagagtttactaaaaaatttaaaatataaatcgaaaacattttttacctaaggtgtgtggacgaaaaattccaggggtgcagatgaaaaaattcaaggggtgcggacgaaaaaatccaaagggtgcagacgagattttcaacggaaaatagcactaaatttttttttcccgggggtgcgcccgcccaccttgggctatatgtatgtccgcccttgtaagtatg

SEQ ID NO: 14 - DNA, 16 bp, Helianthus annuus
  source 1..16: mol_type = other DNA; note = Sequences before the insertion sequence
aaagcttgtaagtatg

SEQ ID NO: 15 - DNA, 16 bp, Helianthus annuus
  source 1..16: mol_type = genomic DNA; note = Sequences after the insertion sequence
ggttctttcatgataa

SEQ ID NO: 16 - DNA, 777 bp, Helianthus annuus
  source 1..777: mol_type = genomic DNA; note = Ha412HOChr04g0188691 gene_HanXRQr2 Chr04g0181821_XM_022179978.2
atgaagatcttcaactgggttcatcgtcgatttcatcacaaatatgaagttagccaagatgtaaagaaagccgaatttactgcgaatgggaaggataatctatcacttcttgaaaatgaaggaatggatggtgtgtttgatggttggaaagaaggcatacttgctattgggacatttgggtttgatccttcgttattgaaagatttcgatcatgaagacgacgacacatacttatgtgaatacacgcgtaaagaattatctattgatcatgatgaggataatggtggagaccaagaagaagaagaagaagaagaagttgagtttccattggtgttcaaagcttgtaagtatggattctttcatgatcaaaaagatgatcacacgcaatgtgatgacgtttgtaaacctaatgatcatgaagactgtgtggatgatcatactgaccagatgaaaaagggaaagaaggctggagaaagaaccactcttgctgatctgtttttggctgattctgataagaacttgttgaacaagaagttgactgatgaagatgatcaagaagtcaaagtccactacatacctgaatccaacataaaacatacttcatatgatgaaagggttgctttgatctctaaaaagaagataacgaaagatgttgctgctcgcccgatcaagaaaattaaccgaatggtgaggaaaatgttaaagaagaagatccatcccgacgtcgaaaatcaaaaggataaatgcaggtttgaagccatgcgcgtacatggatga

SEQ ID NO: 17 - DNA, 777 bp, Helianthus annuus
  source 1..777: mol_type = genomic DNA; note = Ha412HOChr04g0188691 gene_isolated from sunflower plant with lateral flower stalk
atgaagatcttcaactgggttcatcgtcgatttcatcacaaatatgaagttagccaagatgtgaagaaagccgaatttactgcgaatgggaaggacaatctatcacttcttgaaaatgaaggaatggatggtgtgtttgatggttggaaagaaggcatacttgctattgggacatttgggtttgatccttcgttattgaaagatttcgatcatgaagacgacgacacatacttatgtgaatacacgcgtaaagaattatctattgatcatgatgaggataatggtggagaccaagaagaagaagaagaagaagaagttgagtttccattggtgttcaaagcttgtaagtatgggttctttcatgataaaaaagatgatcacacgcaatgtgatgacgtttgtaaacctaatgatcatgaagactgtgtggatgatcatactgaccagatgaaaaagggaaagaaggctggagaaagaaccactcttgctgatctgtttttggctgattctgataagaacttgttgaacaagaagttgactgatgaagatgatcaagaagtcaaagtccactacatacctgaatccaacataaaacatacttcatgtgatgaaagggttgctttgatctctaaaaagaagataacgaaagatgttgctgctcgcccgatcaagaaaattaaccgaatggtgaggaaaatgttgaagaagaagatccatcccgacgtcgaaaatcaaaaggataaatgcaggtttgaagccatgcgcgtacatggatga

SEQ ID NO: 18 - DNA, 777 bp, Helianthus annuus
  source 1..777: mol_type = genomic DNA; note = Ha412HOChr04g0188691 gene_Ha412HOv2.0
atgaagatcttcaactgggttcaccgtcgatttcatcacaaatatgaagttagccaagatgtgaagaaagccgaatttaccgtgaatgggaaggacaatctatcacttcttgaaaatgaaggaatggatggtgtgtttgatggttggaaagaaggcatacttgctattgggacatttgggtttgatccttcgttattgaaagatttcgatcatgaagacgacgacacatacttatgtgaatacacgcgtaaagaattatctattgatcatgatgaggataatggtggagaccaagaagaagaagaagaagaagaagttgagtttccattggtgttcaaagcttgtaagtatgggttctttcatgataaaaaagatgatcacacgcaatgtgatgacgtttgtaaacctaatgatcatgaagactgtgtggatgatcatactgaccagatgaaaaagggaaagaaggctggagaaagaaccactcttgctgatctgtttttggctgattctgataagaacttgttgaacaagaagttgactgatgaagatgatcaagaagtcaaagtccactacatacctgaatccaacataaaacatacttcatatgatgaaagggttgctttgatctctaaaaagaagataacgaaagatgttgctgctcgcccgatcaagaaaattaaccgaatggtgaggaaaatgttaaagaagaagatccatcccgacgtcgaaaatcaaaaggataaatgcaggtttgaagccatgcgcgtacatggatga

SEQ ID NO: 19 - protein, 258 aa, Helianthus annuus
  source 1..258: note = Ha412HOChr04g0188691 _HanXRQr2 Chr04g0181821XP_XP_022035670.1
MKIFNWVHRRFHHKYEVSQDVKKAEFTANGKDNLSLLENEGMDGVFDGWKEGILAIGTFGFDPSLLKDFDHEDDDTYLCEYTRKELSIDHDEDNGGDQEEEEEEEVEFPLVFKACKYGFFHDQKDDHTQCDDVCKPNDHEDCVDDHTDQMKKGKKAGERTTLADLFLADSDKNLLNKKLTDEDDQEVKVHYIPESNIKHTSYDERVALISKKKITKDVAARPIKKINRMVRKMLKKKIHPDVENQKDKCRFEAMRVHG

SEQ ID NO: 20 - protein, 258 aa, Helianthus annuus
  source 1..258: note = Ha412HOChr04g0188691 _isolated from sunflower plant with lateral flower stalk
MKIFNWVHRRFHHKYEVSQDVKKAEFTANGKDNLSLLENEGMDGVFDGWKEGILAIGTFGFDPSLLKDFDHEDDDTYLCEYTRKELSIDHDEDNGGDQEEEEEEEVEFPLVFKACKYGFFHDKKDDHTQCDDVCKPNDHEDCVDDHTDQMKKGKKAGERTTLADLFLADSDKNLLNKKLTDEDDQEVKVHYIPESNIKHTSCDERVALISKKKITKDVAARPIKKINRMVRKMLKKKIHPDVENQKDKCRFEAMRVHG

SEQ ID NO: 21 - protein, 258 aa, Helianthus annuus
  source 1..258: note = Ha412HOChr04g0188691_Ha412HOv2.0
MKIFNWVHRRFHHKYEVSQDVKKAEFTVNGKDNLSLLENEGMDGVFDGWKEGILAIGTFGFDPSLLKDFDHEDDDTYLCEYTRKELSIDHDEDNGGDQEEEEEEEVEFPLVFKACKYGFFHDKKDDHTQCDDVCKPNDHEDCVDDHTDQMKKGKKAGERTTLADLFLADSDKNLLNKKLTDEDDQEVKVHYIPESNIKHTSYDERVALISKKKITKDVAARPIKKINRMVRKMLKKKIHPDVENQKDKCRFEAMRVHG

SEQ ID NO: 22 - DNA, 1632 bp, Helianthus annuus
  source 1..1632: mol_type = genomic DNA; note = Ha412HOChr04g0188691 gene in sunflower plants showing the upward trait in flower stalks
atgaagatcttcaactgggttcatcgtcgatttcatcacaaatatgaagttagccaagatgtgaagaaagccgaatttactgcgaatgggaaggacaatctatcacttcttgaaaatgaaggaatggatggtgtgtttgatggttggaaagaaggcatacttgctattgggacatttgggtttgatccttcgttattgaaagatttcgatcatgaagacgacgacacatacttatgtgaatacacgcgtaaagaattatctattgatcatgatgaggataatggtggagaccaagaagaagaagaagaagaagaagttgagtttccattggtgttcaaagcttgtaagtatgcagtggcggacccaagaatttttccatgggggtgcgaaacatttttaaaaattttaggcccctaggtatataagtaaaaaaatcggttcgtatcgggtcggttcgggtcgggtcatgtaaaacaaaagaaattgcgccataacgtccctactcatggtttctatcacaaacaaattgatgcataagtttatcgctccataaaataatgtttcaattttaattttcaaccctagaaatcgtgtgtaatcagcctaaaaattatctaaacaacataatcaccctaaaaatcatctaaacaaccataaacatcgtcaaaacacatgaaatttcaaacctatttaagaattttgttaccctttggtgtcggacggcggtggttcgcggctgctgatgacgtgctgttgtggtcgatgatcgcttgtaggagacgacccaagagagggagggcgggatgaattctaagggactattgggcttattttaattattatactttgaacttaggttgagtttggttaatgggctagtaattagtgggctaattatgtttaatgaaatagtgggttaaggtattgggtatttgggttaagttgggtagtataagtttatataatttagatagtttttttaattagagtttactaaaaaatttaaaatataaatcgaaaacattttttacctaaggtgtgtggacgaaaaattccaggggtgcagatgaaaaaattcaaggggtgcggacgaaaaaatccaaagggtgcagacgagattttcaacggaaaatagcactaaatttttttttcccgggggtgcgcccgcccaccttgggctatatgtatgtccgcccttgtaagtatgggttctttcatgataaaaaagatgatcacacgcaatgtgatgacgtttgtaaacctaatgatcatgaagactgtgtggatgatcatactgaccagatgaaaaagggaaagaaggctggagaaagaaccactcttgctgatctgtttttggctgattctgataagaacttgttgaacaagaagttgactgatgaagatgatcaagaagtcaaagtccactacatacctgaatccaacataaaacatacttcatgtgatgaaagggttgctttgatctctaaaaagaagataacgaaagatgttgctgctcgcccgatcaagaaaattaaccgaatggtgaggaaaatgttgaagaagaagatccatcccgacgtcgaaaatcaaaaggataaatgcaggtttgaagccatgcgcgtacatggatga

SEQ ID NO: 23 - protein, 138 aa, Helianthus annuus
  source 1..138: note = Ha412HOChr04g0188691 protein in sunflower plants showing the upward trait in flower stalks
MKIFNWVHRRFHHKYEVSQDVKKAEFTANGKDNLSLLENEGMDGVFDGWKEGILAIGTFGFDPSLLKDFDHEDDDTYLCEYTRKELSIDHDEDNGGDQEEEEEEEVEFPLVFKACKYAVADPRIFPWGCETFLKILGP

SEQ ID NO: 24 - DNA, 24 bp, synthetic construct
  source 1..24: mol_type = other DNA; note = Forward primers for detection of Indel marker
agtatgatcatccacacagtcttc

SEQ ID NO: 25 - DNA, 23 bp, synthetic construct
  source 1..23: mol_type = other DNA; note = Reverse primers for detection of Indel marker
cacgcgtaaagaattatctattg

SEQ ID NO: 26 - DNA, 24 bp, synthetic construct
  source 1..24: mol_type = other DNA; note = Forward primer for full-length amplification of Ha412HOChr04g0188691 gene
tcgttcaacaacacatacataaaa

SEQ ID NO: 27 - DNA, 24 bp, synthetic construct
  source 1..24: mol_type = other DNA; note = Reverse primer for full-length amplification of Ha412HOChr04g0188691 gene
tacggatacatgtaatttttgagg